European Patent Application EP 4 538 378 A1, published April 16, 2025. Title: WILD-TYPE-MUTANT Π PROTEIN SWITCHING EXPRESSION SYSTEM CAPABLE OF INCREASING EFFICIENCY OF PREPARING SCREENING-TAG-FREE PLASMID. Applicant: NANJING GENSCRIPT BIOTECH CO., LTD. Application EP 23823135.1, filed June 13, 2023. The sequence listing filed with the application follows.

SEQUENCE LISTING (20 sequences)

SEQ ID NO: 1 - DNA, 204 bp, synthetic construct
  misc_feature 1..204: note = lacO
  source 1..204: mol_type = other DNA
tttacactttatgcttccggctcgtataatgtgtggaattgtgagcggataacaatttcacacaggaaacaggatcgatccatcgatgagcttactccccatccccctgttgacaattaatcatcggctcgtataatgtgtggaattgtgagcggataacaatttcacacaggaaacaggatcagcttactccccatccccctg

SEQ ID NO: 2 - DNA, 918 bp, synthetic construct
  misc_feature 1..918: note = pir116
  source 1..918: mol_type = other DNA
atgagactcaaggtcatgatggacgtgaacaaaaaaacgaaaattcgccaccgaaacgagctaaatcacaccctggctcaacttcctttgcccgcaaagcgagtgatgtatatggcgcttgctcccattgatagcaaagaacctcttgaacgagggcgagttttcaaaattagggctgaagaccttgcagcgctcgccaaaatcaccccatcgcttgcttatcgacaattaaaagagggtggtagattacttggtgccagcaaaatttcgctaagaggggatgatatcattgctttagctaaagagcttaacctgctctttactgctaaaaactcccctgaagagttagatcttaacattattgagtggatagcttattcaaatgatgaaggatacttgtctttaaaattcaccagaaccatagaaccatatatctctagccttattgggaaaaaaaataaattcacaacgcaattgttaacggcaagcttacgcttaagtagccagtattcatcttctctttatcaacttatcaggaagcattactctaattttaagaagaaaaattattttattatttccgttgatgagttaaaggaagagttaatagcttatacttttgataaagatggaaatattgagtacaaataccctgactttcctatttttaaaagggatgtgttaaataaagccattgctgaaattaaaaagaaaacagaaatatcgtttgttggcttcactgttcatgaaaaagaaggaagaaaaattagtaagctgaagttcgaatttgtcgtcgatgaagatgaattttctggcgataaagatgatgaagctttttttatgaatttatctgaagctgatgcagcttttctcaaggtatttgatgaaaccgtacctcccaaaaaagctaaggggtaa

SEQ ID NO: 3 - DNA, 918 bp, synthetic construct
  misc_feature 1..918: note = pirWT
  source 1..918: mol_type = other DNA
atgagactcaaggtcatgatggacgtgaacaaaaaaacgaaaattcgccaccgaaacgagctaaatcacaccctggctcaacttcctttgcccgcaaagcgagtgatgtatatggcgcttgctcccattgatagcaaagaacctcttgaacgagggcgagttttcaaaattagggctgaagaccttgcagcgctcgccaaaatcaccccatcgcttgcttatcgacaattaaaagagggtggtaaattacttggtgccagcaaaatttcgctaagaggggatgatatcattgctttagctaaagagcttaacctgccctttactgctaaaaactcccctgaagagttagatcttaacattattgagtggatagcttattcaaatgatgaaggatacttgtctttaaaattcaccagaaccatagaaccatatatctctagccttattgggaaaaaaaataaattcacaacgcaattgttaacggcaagcttacgcttaagtagccagtattcatcttctctttatcaacttatcaggaagcattactctaattttaagaagaaaaattattttattatttccgttgatgagttaaaggaagagttaatagcttatacttttgataaagatggaaatattgagtacaaataccctgactttcctatttttaaaagggatgtgttaaataaagccattgctgaaattaaaaagaaaacagaaatatcgtttgttggcttcactgttcatgaaaaagaaggaagaaaaattagtaagctgaagttcgaatttgtcgttgatgaagatgaattttctggcgataaagatgatgaagctttttttatgaatttatctgaagctgatgcagcttttctcaaggtatttgatgaaaccgtacctcccaaaaaagctaaggggtaa

SEQ ID NO: 4 - DNA, 498 bp, synthetic construct
  source 1..498: mol_type = other DNA
tgccggtaacgcatccagactgtcatagttattggacacaaaggcatcgcgaggatcttcacgctcacaaatagtgaccagtcccagaccttgcgggaattcaaccggcacatctttcattgagtgtacggcgatatcggcgcgattttcgaggagcgcgacttccagctcttttacaaataagccttttccgcctactttcgccagcggcgtatcaagaatcacatcgccgcgcgtcaccatcggtaccagttcaacgaccaggcccggatggctcgccatcaacttgtctttgacatagtgtgcctgccagagtgcaagtgggctttggcgtgtggcaattcttaaaacattgtctaacatgcttgttaccgtcattatcatccgtggtccatcctaacatccttgccagagtgatgtcagtgttgtggtgaaacgtagacgcctgcgcaaaccgtaaaatgaggtctggcagtggatcctgacaggcgtttcacg

SEQ ID NO: 5 - DNA, 491 bp, synthetic construct
  source 1..491: mol_type = other DNA
tgctacacttgtatgtagcgcatctttctttacggtcaatcagcaaggtgttaaattgatcacgttttagaccattttttcgtcgtgaaactaaaaaaaccaggcgcgaaaagtggtaacggttacctttgacatacgaaatatcccgaatgccgcgtgttaccgttgatgttggcggaatcacagtcatgacgggtagcaaatcaggcgatacgtcttgtacctctatattgagactctgaaacagagactggatgccataaatcaattgcgtgtggatcgcgcgcttgctgctatggggcctgcattccaacaggtctacagtctactgccgacattgttgcactatcaccatccgctaatgccgggttaccttgatggtaacgttcccaaaggcatttgcctttacacgcctgatgaaactcaacgccactacctgaacgagcttgaactgtatcgtggaatgtcagtacaggatccgccgaaaggtg

SEQ ID NO: 6 - DNA, 25 bp, synthetic construct
  misc_feature 1..25: note = C4241GG050-1JJFH
  source 1..25: mol_type = other DNA
ttagtccggctacggcaagaatgat

SEQ ID NO: 7 - DNA, 25 bp, synthetic construct
  misc_feature 1..25: note = C4241GG050-1JJRH
  source 1..25: mol_type = other DNA
gctgacttccacacccagcgaggcg

SEQ ID NO: 8 - DNA, 389 bp, synthetic construct
  misc_feature 1..389: note = oriR6K
  source 1..389: mol_type = other DNA
tgtcagccgttaagtgttcctgtgtcactcaaaattgctttgagaggctctaagggcttctcagtgcgttacatccctggcttgttgtccacaaccgttaaaccttaaaagctttaaaagccttatatattcttttttttcttataaaacttaaaaccttagaggctatttaagttgctgatttatattaattttattgttcaaacatgagagcttagtacgtgaaacatgagagcttagtacgttagccatgagagcttagtacgttagccatgagggtttagttcgttaaacatgagagcttagtacgttaaacatgagagcttagtacgtgaaacatgagagcttagtacgtactatcaacaggttgaactgctgatcttcagatc

SEQ ID NO: 9 - DNA, 20 bp, synthetic construct
  misc_feature 1..20: note = gRNA
  source 1..20: mol_type = other DNA
ttgtaataaggaatttacag

SEQ ID NO: 10 - DNA, 34 bp, synthetic construct
  misc_feature 1..34: note = Lox71
  source 1..34: mol_type = other DNA
taccgttcgtataatgtatgctatacgaagttat

SEQ ID NO: 11 - DNA, 34 bp, synthetic construct
  misc_feature 1..34: note = Lox66
  source 1..34: mol_type = other DNA
ataacttcgtataatgtatgctatacgaacggta

SEQ ID NO: 12 - DNA, 3369 bp, synthetic construct
  misc_feature 1..3369: note = pMF5-loxp-RFP
  source 1..3369: mol_type = other DNA
ttctcatgtttgacagcttatcatcgataagctttaatgcggtagtttatcacagttaaattgctaacgcagtcaggcaccgtgtatggaagccggcggcacctcgctaacggattcaccactccaagaattggagccaatcaattcttgcggagaactgtgaatgcgcaaaccaacccttggcagaacatatccatcgcgtccgccatctccagcagccgcacgcggcgcatctcgggcagcgttgggtcctggccacgggtgcgcatgatcgtgctcctgtcgttgaggacccggctaggctggcggggttgccttactggttagcagaatgaatcaccgatacgcgagcgaacgtgaagcgactgctgctgcaaaacgtctgcgacctgagcaacaacatgaatggtcttcggtttccgtgtttcgtaaagtctggaaacgcggaagtcagcgccctgcaccattatgttccggatctgcatcgcaggatgctgctggctaccctgtggaacacctacatctgtattaacgaagcgctggcattgaccctgagtgatttttctctggtcccgccgcatccataccgccagttgtttaccctcacaacgttccagtaaccgggcatgttcatcatcagtaacccgtatcgtgagcatcctctctcgtttcatcggtatcattacccccatgaacagaaatcccccttacacggaggcatcaataacttcgtataatgtatgctatacgaacggtactgcagtgtcagccgttaagtgttcctgtgtcactcaaaattgctttgagaggctctaagggcttctcagtgcgttacatccctggcttgttgtccacaaccgttaaaccttaaaagctttaaaagccttatatattcttttttttcttataaaacttaaaaccttagaggctatttaagttgctgatttatattaattttattgttcaaacatgagagcttagtacgtgaaacatgagagcttagtacgttagccatgagagcttagtacgttagccatgagggtttagttcgttaaacatgagagcttagtacgttaaacatgagagcttagtacgtgaaacatgagagcttagtacgtactatcaacaggttgaactgctgatcttcagatcggtacccaatacgcaaaccgcctctccccgcgcgttggccgattcattaatgcagctggcacgacaggtttcccgactggaaagcgggcagtgagcgcaacgcaattaatgtgagttagctcactcattaggcaccccaggctttacactttatgcttccggctcgtatgttgtgtggaattgtgagcggataacaatttcacacatactagagaaagaggagaaatactagatggcttcctccgaagacgttatcaaagagttcatgcgtttcaaagttcgtatggaaggttccgttaacggtcacgagttcgaaatcgaaggtgaaggtgaaggtcgtccgtacgaaggtacccagaccgctaaactgaaagttaccaaaggtggtccgctgccgttcgcttgggacatcctgtccccgcagttccagtacggttccaaagcttacgttaaacacccggctgacatcccggactacctgaaactgtccttcccggaaggtttcaaatgggaacgtgttatgaacttcgaagacggtggtgttgttaccgttacccaggactcctccctgcaagacggtgagttcatctacaaagttaaactgcgtggtaccaacttcccgtccgacggtccggttatgcagaaaaaaaccatgggttgggaagcttccaccgaacgtatgtacccggaagacggtgctctgaaaggtgaaatcaaaatgcgtctgaaactgaaagacggtggtcactacgacgctgaagttaaaaccacctacatggctaaaaaaccggttcagctgccgggtgcttacaaaaccgacatcaaactggacatcacctcccacaacgaagactacaccatcgttgaacagtacgaacgtgctgaaggtcgtcactccaccggtgcttaataacgctgatagtgctagtgtagatcgctactagagccaggcatcaaataaaacgaaaggctcagtcgaaagactgggcctttcgttttatctgttgtttgtcggtgaacgctctctactagagtcacactggctcaccttcgggtgggcctttctgcgtttatagtcgactcgagcggccagtcgacgcatgctaccgttcgtataatgtatgctatacgaagttattgatcttttctacggggtctgacgctcagtggaacgaaaactcacgttaagggattttggtcatgagattatcaaaaaggatcttcacctagatccttttaaattaaaaatgaagttttaaatcaatctaaagtatatatgagtaaacttggtctgacagttagaaaaactcatcgagcatcaaatgaaactgcaatttattcatatcaggattatcaataccatatttttgaaaaagccgtttctgtaatgaaggagaaaactcaccgaggcagttccataggatggcaagatcctggtatcggtctgcgattccgactcgtccaacatcaatacaacctattaatttcccctcgtcaaaaataaggttatcaagtgagaaatcaccatgagtgacgactgaatccggtgagaatggcaaaagtttatgcatttctttccagacttgttcaacaggccagccattacgctcgtcatcaaaatcactcgcatcaaccaaaccgttattcattcgtgattgcgcctgagcgagacgaaatacgcgatcgctgttaaaaggacaattacaaacaggaatcgaatgcaaccggcgcaggaacactgccagcgcatcaacaatattttcacctgaatcaggatattcttctaatacctggaatgctgttttcccggggatcgcagtggtgagtaaccatgcatcatcaggagtacggataaaatgcttgatggtcggaagaggcataaattccgtcagccagtttagtctgaccatctcatctgtaacatcattggcaacgctacctttgccatgtttcagaaacaactctggcgcatcgggcttcccatacaatcgatagattgtcgcacctgattgcccgacattatcgcgagcccatttatacccatataaatcagcatccatgttggaatttaatcgcggcctagagcaagacgtttcccgttgaatatggctcatcacatttccccgaaaagtgccacctgacgtctaagaaaccattattatcatgacattaacctataaaaataggcgtatcacgaggccctttcgtcttcaagaa

SEQ ID NO: 13 - DNA, 1050 bp, synthetic construct
  misc_feature 1..1050: note = Cre
  source 1..1050: mol_type = other DNA
caccatcaccatcaccatatgtccaatttactgaccgtacaccaaaatttgcctgcattaccggtcgatgcaacgagtgatgaggttcgcaagaacctgatggacatgttcagggatcgccaggcgttttctgagcatacctggaaaatgcttctgtccgtttgccggtcgtgggcggcatggtgcaagttgaataaccggaaatggtttcccgcagaacctgaagatgttcgcgattatcttctatatcttcaggcgcgcggtctggcagtaaaaactatccagcaacatttgggccagctaaacatgcttcatcgtcggtccgggctgccacgaccaagtgacagcaatgctgtttcactggttatgcggcggatccgaaaagaaaacgttgatgccggtgaacgtgcaaaacaggctctagcgttcgaacgcactgatttcgaccaggttcgttcactcatggaaaatagcgatcgctgccaggatatacgtaatctggcatttctggggattgcttataacaccctgttacgtatagccgaaattgccaggatcagggttaaagatatctcacgtactgacggtgggagaatgttaatccatattggcagaacgaaaacgctggttagcaccgcaggtgtagagaaggcacttagcctgggggtaactaaactggtcgagcgatggatttccgtctctggtgtagctgatgatccgaataactacctgttttgccgggtcagaaaaaatggtgttgccgcgccatctgccaccagccagctatcaactcgcgccctggaagggatttttgaagcaactcatcgattgatttacggcgctaaggatgactctggtcagagatacctggcctggtctggacacagtgcccgtgtcggagccgcgcgagatatggcccgcgctggagtttcaataccggagatcatgcaagctggtggctggaccaatgtaaatattgtcatgaactatatccgtaacctggatagtgaaacaggggcaatggtgcgcctgctggaagatggcgattaa

SEQ ID NO: 14 - DNA, 50 bp, synthetic construct
  misc_feature 1..50: note = lacI-F
  source 1..50: mol_type = other DNA
aagtatatatgagtaaacttggtctgacaggacaccatcgaatggtgcaa

SEQ ID NO: 15 - DNA, 56 bp, synthetic construct
  misc_feature 1..56: note = lacI-R
  source 1..56: mol_type = other DNA
gttcacgtccatcatgaccttgagtctcatctcgagtcactgcccgctttccagtc

SEQ ID NO: 16 - DNA, 20 bp, synthetic construct
  misc_feature 1..20: note = pir-F
  source 1..20: mol_type = other DNA
atgagactcaaggtcatgat

SEQ ID NO: 17 - DNA, 37 bp, synthetic construct
  misc_feature 1..37: note = pir-R
  source 1..37: mol_type = other DNA
tttcatttgatgctcgatgagtttttctaaggttctt

SEQ ID NO: 18 - DNA, 20 bp, synthetic construct
  misc_feature 1..20: note = R6K WT-loxp-F
  source 1..20: mol_type = other DNA
ttagaaaaactcatcgagca

SEQ ID NO: 19 - DNA, 20 bp, synthetic construct
  misc_feature 1..20: note = R6K WT-loxp-R
  source 1..20: mol_type = other DNA
ctgtcagaccaagtttactc

SEQ ID NO: 20 - DNA, 78 bp, synthetic construct
  misc_feature 1..78: note = PlacIq
  source 1..78: mol_type = other DNA
gacaccatcgaatggtgcaaaacctttcgcggtatggcatgatagcgcccggaagagagtcaattcagggtggtgaat